European Patent Application EP 4 474 392 A1, published December 11, 2024. Title: BROADLY NEUTRALIZING ANTIBODIES TARGETING THE CD4 BINDING SITE ON HIV ENV. Applicant: Universität zu Köln. The sequence listing filed with the application follows.

SEQUENCE LISTING (8 sequences)

SEQ ID NO: 1 - protein, 19 aa, synthetic construct
  source 1..19: note = VH CDR 1
DSFTVYRPRLSAYFIGEFN

SEQ ID NO: 2 - protein, 8 aa, synthetic construct
  source 1..8: note = VH CDR 2
VNIFRGAV

SEQ ID NO: 3 - protein, 15 aa, synthetic construct
  source 1..15: note = VH CDR3
AWDKNVDDNPWRLDS

SEQ ID NO: 4 - protein, 6 aa, synthetic construct
  source 1..6: note = VL CDR 1
QDVGWA

SEQ ID NO: 5 - skipped

SEQ ID NO: 6 - protein, 5 aa, synthetic construct
  source 1..5: note = VL CDR 3
QVFDS

SEQ ID NO: 7 - protein, 133 aa, synthetic construct
  source 1..133: note = VH chain
SVRLDQSGTAVKKPGASVRVSCRAPDSFTVYRPRLSAYFIGEFNIHWLRQAPGQGLEWLGFVNIFRGAVKYSSRFQGRITITRDTSSETSYLDLGALKADDTATYYCAWDKNVDDNPWRLDSWGQGTLVIVSS

SEQ ID NO: 8 - protein, 103 aa, synthetic construct
  source 1..103: note = VL chain
YIQVTQSPSSLSASIGDTITVACEVSQDVGWAVNWYHQRPGRPPYNLIYTAHNLAPGVASRFRGSRVGTYFTLTINNLLPEDVGTYYCQVFDSFAPGGTRVDL